European Patent Specification EP 3 489 677 B1, published January 18, 2023. Title: Method of Detecting Allergen. Applicant: NISSHIN SEIFUN GROUP INC. The sequence listing filed with the application follows.

SEQUENCE LISTING (26 sequences)

SEQ ID NO: 1 - protein, 9 aa, Fagopyrum esculentum
VQVVGDEGR

SEQ ID NO: 2 - protein, 9 aa, Fagopyrum esculentum
SVFDDNVQR

SEQ ID NO: 3 - protein, 15 aa, Fagopyrum esculentum
GQILVVPQGFAVVLK

SEQ ID NO: 4 - protein, 9 aa, Fagopyrum esculentum
EGLEWVELK

SEQ ID NO: 5 - protein, 9 aa, Fagopyrum esculentum
NFFLAGQSK

SEQ ID NO: 6 - protein, 7 aa, Fagopyrum esculentum
GFIVQAR

SEQ ID NO: 7 - protein, 13 aa, Fagopyrum esculentum
NDDNAITSPIAGK

SEQ ID NO: 8 - protein, 10 aa, Marsupenaeus japonicus
IQLLEEDLER

SEQ ID NO: 9 - protein, 9 aa, Marsupenaeus japonicus
MDALENQLK

SEQ ID NO: 10 - protein, 8 aa, Marsupenaeus japonicus
FLAEEADR

SEQ ID NO: 11 - protein, 9 aa, Marsupenaeus japonicus
IVELEEELR

SEQ ID NO: 12 - protein, 10 aa, Marsupenaeus japonicus
LAMVEADLER

SEQ ID NO: 13 - protein, 12 aa, Bos taurus
FFVAPFPEVFGK

SEQ ID NO: 14 - protein, 10 aa, Bos taurus
YLGYLEQLLR

SEQ ID NO: 15 - protein, 11 aa, Bos taurus
NAVPITPTLNR

SEQ ID NO: 16 - protein, 9 aa, Bos taurus
VLVLDTDYK

SEQ ID NO: 17 - protein, 11 aa, Bos taurus
TPEVDDEALEK

SEQ ID NO: 18 - protein, 12 aa, Gallus gallus
YPILPEYLQCVK

SEQ ID NO: 19 - protein, 16 aa, Gallus gallus
ELINSWVESQTNGIIR

SEQ ID NO: 20 - protein, 13 aa, Gallus gallus
LTEWTSSNVMEER

SEQ ID NO: 21 - protein, 12 aa, Gallus gallus
HIATNAVLFFGR

SEQ ID NO: 22 - protein, 13 aa, Arachis hypogaea
DLAFPGSGEQVEK

SEQ ID NO: 23 - protein, 14 aa, Arachis hypogaea
VLLEENAGGEQEER

SEQ ID NO: 24 - protein, 13 aa, Arachis hypogaea
SPDIYNPQAGSLK

SEQ ID NO: 25 - protein, 183 aa, Fagopyrum esculentum
LKFRQNVNRPSRADVFNPRAGRINTVDSNNLPILEFIQLSAQHVVLYKNAILGPRWNLNAHSALYVTRGEGRVQVVGDEGRSVFDDNVQRGQILVVPQGFAVVLKAGREGLEWVELKNDDNAITSPIAGKTSVLRAIPVEVLANSYDISTKEAFRLKNGRQEVEVFRPFQSRDEKERERFSIV

SEQ ID NO: 26 - protein, 284 aa, Marsupenaeus japonicus
MDAIKKKMQAMKLEKDNAMDRADTLEQQNKEANNRAEKSEEEVHNLQKRMQQLENDLDQVQESLLKANIQLVEKDKALSNAEGEVAALNRRIQLLEEDLERSEERLNTATTKLAEASQAADESERMRKVLENRSLSDEERMDALENQLKEARFLAEEADRKYDEVARKLAMVEADLERAEERAETGESKIVELEEELRVVGNNLKSLEVSEEKANQREEAYKEQIKTLTNKLKAAEARAEFAERSVQKLQKEVDRLEDELVNEKEKYKSITDELDQTFSELSGY